European Patent Specification EP 3 778 885 B1, published March 8, 2023. Title: COMPOSITIONS OF ENGINEERED HUMAN ARGINASES AND METHODS FOR TREATING CANCER. Applicant: AERase, Inc. Application UNKNOWN. The sequence listing filed with the application follows.

SEQUENCE LISTING (12 sequences)

SEQ ID NO: 1 - DNA, 1044 bp, Artificial Sequence
  Synthetic primer
gatataccatgggttcttctcaccatcatcaccaccacagctctggcgagaacctgtacttccagtctgcgaagagccgtacgatcggcattattggtgcgccgttctctaaaggtcagccacgcggtggtgtggaagagggtccgacggttctgcgtaaggccggtttattagaaaagctgaaagagcaggagtgcgacgttaaggactacggtgacttaccattcgcggacatcccgaatgatagcccgttccaaatcgttaagaatccgcgctctgtgggtaaagcaagcgagcagttagcaggtaaggtggccgaggtcaagaaaaacggtcgtattagcctggttttaggcggtgatcatagcttagcaattggctctatctctggtcatgcccgtgtgcacccagatttaggtgtcatttgggttgacgcccatacggatatcaatacgccattaacgaccaccagcggcaatctgcatggccagccggttagcttcttactgaaggagctgaagggtaaaattccagatgttccgggctttagctgggtcacgccatgtatttctgccaaggatatcgtgtacattggcttacgtgacgtcgacccaggtgagcactacatcttaaagaccctgggtatcaagtatttcagcatgacggaagtggaccgcttaggcatcggcaaggtgatggaggagacgctgagctatctgctgggccgtaagaaacgtccaatccatctgagcttcgatgttgacggcttagacccgagctttacgccagccaccggcacgccggtcgttggtggtttaacgtatcgcgaaggcctgtatatcacggaggaaatctataagacgggtttactgagcggtctggacattatggaggttaatccaagcttaggtaagacgccggaagaagttacccgtaccgttaacacggcggtcgcgatcacgttagcatgtttcggtttagcccgcgagggcaaccataaaccaattgattatctgaatccaccgaagtgaggatccgaattcg

SEQ ID NO: 2 - DNA, 1080 bp, Artificial Sequence
  Synthetic primer
gatataccatgggcagcagccatcatcaccaccatcacagctctggtgaaaacttatacttccaaagcgtccatagcgtcgcagtgattggtgccccgtttagccaaggtcaaaaacgcaagggtgttgaacatggtccggcagcgatccgcgaagcaggtttaatgaagcgtttaagcagcttaggctgtcacttaaaggatttcggtgatttaagctttacgccggtcccaaaggatgatttatacaataatctgatcgttaacccacgctctgtgggtctggcgaaccaggagctggcggaggtcgtgtctcgtgcagtcagcgacggttatagctgcgttacgctgggcggtgatcatagcttagccattggtacgatttctggtcatgcccgccattgcccggatctgtgtgttgtgtgggttgatgcgcacgcggatatcaatacgccactgaccacgtctagcggtaatttacacggccagccggttagcttcttattacgtgagctgcaagacaaggtcccgcagttaccaggcttctcttggatcaaaccatgtatcagcagcgcatctattgtctacattggcctgcgtgatgtcgacccaccggagcacttcatcctgaagaattatgacatccagtatttcagcatgcgtgacatcgaccgtctgggtatccaaaaagttatggagcgcacgttcgatctgttaatcggcaagcgccagcgtccgattcacctgagctttgacattgacgcctttgacccgaccctggccccagcaacgggcacgccagtggttggtggtttaacctaccgtgagggtatgtatattgcagaagagatccataataccggcctgttatctgccctggatctggttgaagtcaatccgcagctggcaacctctgaggaggaagcgaagacgaccgccaacctggcggtggacgtcatcgcctcttctttcggccagacgcgtgaaggtggccatatcgtgtatgaccaattaccaacgccatctagcccggacgaatctgagaaccaagcacgtgtccgtatttgaggatccgaattcg

SEQ ID NO: 3 - DNA, 31 bp, Artificial Sequence
  Synthetic primer
  misc_feature (15)..(16): n is a, c, g, or t
cgatcacgttagcannsttcggtttagcccg

SEQ ID NO: 4 - DNA, 31 bp, Artificial Sequence
  Synthetic primer
  misc_feature (16)..(17): n is a, c, g, or t
cgggctaaaccgaasnntgctaacgtgatcg

SEQ ID NO: 5 - DNA, 48 bp, Artificial Sequence
  Synthetic primer
gatataccatgggttcttctcaccatcatcaccaccacagctctggcg

SEQ ID NO: 6 - DNA, 41 bp, Artificial Sequence
  Synthetic primer
cgaattcggatcctcacttcggtggattcagataatcaatt

SEQ ID NO: 7 - DNA, 27 bp, Artificial Sequence
  Synthetic primer
  misc_feature (14)..(15): n is a, c, g, or t
cattggcttacgtnnsgtcgacccagg

SEQ ID NO: 8 - DNA, 27 bp, Artificial Sequence
  Synthetic primer
  misc_feature (13)..(14): n is a, c, g, or t
cctgggtcgacsnnacgtaagccaatg

SEQ ID NO: 9 - DNA, 31 bp, Artificial Sequence
  Synthetic primer
  misc_feature (16)..(17): n is a, c, g, or t
cgtccaatccatctgnnsttcgatgttgacg

SEQ ID NO: 10 - DNA, 31 bp, Artificial Sequence
  Synthetic primer
  misc_feature (15)..(16): n is a, c, g, or t
cgtcaacatcgaasnncagatggattggacg

SEQ ID NO: 11 - DNA, 34 bp, Artificial Sequence
  Synthetic primer
ggtttaacgtatcgccagggcctgtatatcacgg

SEQ ID NO: 12 - DNA, 34 bp, Artificial Sequence
  Synthetic primer
ccgtgatatacaggccctggcgatacgttaaacc